European Patent Application EP 4 137 574 A1, published February 22, 2023. Title: Method for removing color of protein preparations. Applicant: ONO PHARMACEUTICAL CO., LTD. The sequence listing filed with the application follows.

SEQUENCE LISTING (19 sequences)

SEQ ID NO: 1 - protein, 456 aa, Homo sapiens
QVQLVQSGSELKQPGASVKVSCKASGYTFTHYGLHWVRQAPGQGLEWMGWLNTNTENPTFAQGFTGRFVFSLDTSVTTAYLQISSLKAEDTAVYYCARGDMVVPTTIWNYYHFMDVWGNGTLVTVSSASTKGPSVFPLAPSSKSTSGGTAALGCLVKDYFPEPVTVSWNSGALTSGVHTFPAVLQSSGLYSLSSVVTVPSSSLGTQTYICNVNHKPSNTKVDKRVEPKSCDKTHTCPPCPAPELGRGPSVFLFPPKPKDTLMISRTPEVTCVVVDVSHEDPEVKFNWYVDGVEVHNAKTKPREEQYNSTYRVVSVLTVLHQDWLNGKEYKCKVSNKALPAPIEKTISKAKGQPREPQVYTDPPSREEMTKNQVSLTCEVKGFYPSDIAVEWESNGQPENNYKTTPPVLDSDGSFFLYSKLTVDKSRWQQGNVFSCSVMHEALHNHYTQKSLSLSPG

SEQ ID NO: 2 - protein, 456 aa, Homo sapiens
QVQLVQSGSELKQPGVSVKVSCKASGYTFTHYGLHWVRQAPGQGLEWMGWINTNTGNPTYAQGFTGRFVFSLDTSVSTAYLQISSLKAEDTAVYYCARGDLVVPTTIWNYYHYMEVWGKGTLVTVSSASTKGPSVFPLAPSSKSTSGGTAALGCLVKDYFPEPVTVSWNSGALTSGVHTFPAVLQSSGLYSLSSVVTVPSSSLGTQTYICNVNHKPSNTKVDKRVEPKSCDKTHTCPPCPAPELGRGPSVFLFPPKPKDTLMISRTPEVTCVVVDVSHEDPEVKFNWYVDGVEVHNAKTKPREEQYNSTYRVVSVLTVLHQDWLNGKEYKCKVSNKALPAPIEKTISKAKGQPREPQVYTDPPSREEMTKNQVSLTCEVKGFYPSDIAVEWESNGQPENNYKTTPPVLDSDGSFFLYSKLTVDKSRWQQGNVFSCSVMHEALHNHYTQKSLSLSPG

SEQ ID NO: 3 - protein, 456 aa, Homo sapiens
QVQLVQSGSELKKPGASVMVSCKASGYTFTHYALHWVRQAPGQGLEWMGWLNTNTENPTYAQGFTGRFVFSLDTSVTTAYLQINSLKAEDTAVYYCARGDMVVPTTIWNYYYYMDVWGKGTTVTVSSASTKGPSVFPLAPSSKSTSGGTAALGCLVKDYFPEPVTVSWNSGALTSGVHTFPAVLQSSGLYSLSSVVTVPSSSLGTQTYICNVNHKPSNTKVDKRVEPKSCDKTHTCPPCPAPELGRGPSVFLFPPKPKDTLMISRTPEVTCVVVDVSHEDPEVKFNWYVDGVEVHNAKTKPREEQYNSTYRVVSVLTVLHQDWLNGKEYKCKVSNKALPAPIEKTISKAKGQPREPQVYTDPPSREEMTKNQVSLTCEVKGFYPSDIAVEWESNGQPENNYKTTPPVLDSDGSFFLYSKLTVDKSRWQQGNVFSCSVMHEALHNHYTQKSLSLSPG

SEQ ID NO: 4 - protein, 456 aa, Homo sapiens
QVQLVQSGSELKQPGASVKVSCKASGYTFTHYALHWLRQAPGQGLEWMGWLNTNTENPTFAQGFTGRFVFSLDTSVTTAYLQISSLKAEDTAVYYCARGDMVVPTTIWNYYHFMDVWGNGTTVTVSSASTKGPSVFPLAPSSKSTSGGTAALGCLVKDYFPEPVTVSWNSGALTSGVHTFPAVLQSSGLYSLSSVVTVPSSSLGTQTYICNVNHKPSNTKVDKRVEPKSCDKTHTCPPCPAPELGRGPSVFLFPPKPKDTLMISRTPEVTCVVVDVSHEDPEVKFNWYVDGVEVHNAKTKPREEQYNSTYRVVSVLTVLHQDWLNGKEYKCKVSNKALPAPIEKTISKAKGQPREPQVYTDPPSREEMTKNQVSLTCEVKGFYPSDIAVEWESNGQPENNYKTTPPVLDSDGSFFLYSKLTVDKSRWQQGNVFSCSVMHEALHNHYTQKSLSLSPG

SEQ ID NO: 5 - protein, 456 aa, Homo sapiens
QVQLVQSGSELKQPGASVKVSCKASGYTFTHYALHWLRQAPGQGLEWMGWLNTNTENPTFAQGFTGRFVFSLDTSVTTAYLQISSLKAEDTAVYYCARGDMVVPTTIWNYYHFMDVWGQGTTVTVSSASTKGPSVFPLAPSSKSTSGGTAALGCLVKDYFPEPVTVSWNSGALTSGVHTFPAVLQSSGLYSLSSVVTVPSSSLGTQTYICNVNHKPSNTKVDKRVEPKSCDKTHTCPPCPAPELGRGPSVFLFPPKPKDTLMISRTPEVTCVVVDVSHEDPEVKFNWYVDGVEVHNAKTKPREEQYNSTYRVVSVLTVLHQDWLNGKEYKCKVSNKALPAPIEKTISKAKGQPREPQVYTDPPSREEMTKNQVSLTCEVKGFYPSDIAVEWESNGQPENNYKTTPPVLDSDGSFFLYSKLTVDKSRWQQGNVFSCSVMHEALHNHYTQKSLSLSPG

SEQ ID NO: 6 - protein, 447 aa, Homo sapiens
QVQLVQSGGGVVQPGRSLRLSCVASGFTFSSYGMHWVRQAPGKGLEWVAQIWYNARKQEYSDSVKGRFTISRDNSKNTLYLQMNSLRAEDTAVYYCTRGTGYNWFDPWGQGTLVTVSSASTKGPSVFPLAPSSKSTSGGTAALGCLVKDYFPEPVTVSWNSGALTSGVHTFPAVLQSSGLYSLSSVVTVPSSSLGTQTYICNVNHKPSNTKVDKRVEPKSCDKTHTCPPCPAPELGRGPSVFLFPPKPKDTLMISRTPEVTCVVVDVSHEDPEVKFNWYVDGVEVHNAKTKPREEQYNSTYRVVSVLTVLHQDWLNGKEYKCKVSNKALPAPIEKTISKAKGQPREPQVYTKPPSREEMTKNQVSLKCLVKGFYPSDIAVEWESNGQPENNYKTTPPVLDSDGSFFLYSKLTVDKSRWQQGNVFSCSVMHEALHNHYTQKSLSLSPG

SEQ ID NO: 7 - protein, 214 aa, Homo sapiens
DIQMTQSPSSLSASVGDRVTITCRASQSISSYLNWYQQKPGKAPKLLIYAASSLQSGVPSRFSGSGSGTDFTLTISSLQPEDFATYYCQQSYSTPPTFGQGTKVEIKRTVAAPSVFIFPPSDEQLKSGTASVVCLLNNFYPREAKVQWKVDNALQSGNSQESVTEQDSKDSTYSLSSTLTLSKADYEKHKVYACEVTHQGLSSPVTKSFNRGEC

SEQ ID NO: 8 - protein, 329 aa, Homo sapiens
ASTKGPSVFPLAPSSKSTSGGTAALGCLVKDYFPEPVTVSWNSGALTSGVHTFPAVLQSSGLYSLSSVVTVPSSSLGTQTYICNVNHKPSNTKVDKRVEPKSCDKTHTCPPCPAPELGRGPSVFLFPPKPKDTLEISRTPEVTCVVVDVSHEDPEVKFNWYVDGVEVHNAKTKPREEQYNSTYRVVSVLTVLHQDWLNGKEYKCKVSNKALPAPIEKTISKAKGQPREPQVYTDPPSREEMTKNQVSLTCEVKGFYPSDIAVEWESNGQPENNYKTTPPVLDSDGSFFLYSKLTVDKSRWQQGNVFSCSVMHEALHNHYTQKSLSLSPG

SEQ ID NO: 9 - protein, 329 aa, Homo sapiens
ASTKGPSVFPLAPSSKSTSGGTAALGCLVKDYFPEPVTVSWNSGALTSGVHTFPAVLQSSGLYSLSSVVTVPSSSLGTQTYICNVNHKPSNTKVDKRVEPKSCDKTHTCPPCPAPELGRGPSVFLFPPKPKDTLPISRTPEVTCVVVDVSHEDPEVKFNWYVDGVEVHNAKTKPREEQYNSTYRVVSVLTVLHQDWLNGKEYKCKVSNKALPAPIEKTISKAKGQPREPQVYTDPPSREEMTKNQVSLTCEVKGFYPSDIAVEWESNGQPENNYKTTPPVLDSDGSFFLYSKLTVDKSRWQQGNVFSCSVMHEALHNHYTQKSLSLSPG

SEQ ID NO: 10 - protein, 329 aa, Homo sapiens
ASTKGPSVFPLAPSSKSTSGGTAALGCLVKDYFPEPVTVSWNSGALTSGVHTFPAVLQSSGLYSLSSVVTVPSSSLGTQTYICNVNHKPSNTKVDKRVEPKSCDKTHTCPPCPAPELGRGPSVFLFPPKPKDTLRISRTPEVTCVVVDVSHEDPEVKFNWYVDGVEVHNAKTKPREEQYNSTYRVVSVLTVLHQDWLNGKEYKCKVSNKALPAPIEKTISKAKGQPREPQVYTDPPSREEMTKNQVSLTCEVKGFYPSDIAVEWESNGQPENNYKTTPPVLDSDGSFFLYSKLTVDKSRWQQGNVFSCSVMHEALHNHYTQKSLSLSPG

SEQ ID NO: 11 - protein, 329 aa, Homo sapiens
ASTKGPSVFPLAPSSKSTSGGTAALGCLVKDYFPEPVTVSWNSGALTSGVHTFPAVLQSSGLYSLSSVVTVPSSSLGTQTYICNVNHKPSNTKVDKRVEPKSCDKTHTCPPCPAPELGRGPSVFLFPPKPKDTLDISRTPEVTCVVVDVSHEDPEVKFNWYVDGVEVHNAKTKPREEQYNSTYRVVSVLTVLHQDWLNGKEYKCKVSNKALPAPIEKTISKAKGQPREPQVYTDPPSREEMTKNQVSLTCEVKGFYPSDIAVEWESNGQPENNYKTTPPVLDSDGSFFLYSKLTVDKSRWQQGNVFSCSVMHEALHNHYTQKSLSLSPG

SEQ ID NO: 12 - protein, 329 aa, Homo sapiens
ASTKGPSVFPLAPSSKSTSGGTAALGCLVKDYFPEPVTVSWNSGALTSGVHTFPAVLQSSGLYSLSSVVTVPSSSLGTQTYICNVNHKPSNTKVDKRVEPKSCDKTHTCPPCPAPELGRGPSVFLFPPKPKDTLMISRTPEVTCVVVDVSHEDPEVKFNWYVDGVEVHNAKTKPREEQYNSTYRVVSVLTVLHQDWLNGKEYKCKVSNKALPAPIEKTISKAKGQPREPQVYTDPPSREEMTKNQVSLTCEVKGFYPSDIAVEWESNGQPENNYKTTPPVLDSDGSFFLYSKLTVDKSRWQQGNVFSCSVMHEALHLHYTQKSLSLSPG

SEQ ID NO: 13 - protein, 329 aa, Homo sapiens
ASTKGPSVFPLAPSSKSTSGGTAALGCLVKDYFPEPVTVSWNSGALTSGVHTFPAVLQSSGLYSLSSVVTVPSSSLGTQTYICNVNHKPSNTKVDKRVEPKSCDKTHTCPPCPAPELGRGPSVFLFPPKPKDTLMISRTPEVTCVVVDVSHEDPEVKFNWYVDGVEVHNAKTKPREEQYNSTYRVVSVLTVLHQDWLNGKEYKCKVSNKALPAPIEKTISKAKGQPREPQVYTDPPSREEMTKNQVSLTCEVKGFYPSDIAVEWESNGQPENNYKTTPPVLDSDGSFFLYSKLTVDKSRWQQGNVFSCSVMHEALHNHYTEKSLSLSPG

SEQ ID NO: 14 - protein, 329 aa, Homo sapiens
ASTKGPSVFPLAPSSKSTSGGTAALGCLVKDYFPEPVTVSWNSGALTSGVHTFPAVLQSSGLYSLSSVVTVPSSSLGTQTYICNVNHKPSNTKVDKRVEPKSCDKTHTCPPCPAPELGRGPSVFLFPPKPKDTLEISRTPEVTCVVVDVSHEDPEVKFNWYVDGVEVHNAKTKPREEQYNSTYRVVSVLTVLHQDWLNGKEYKCKVSNKALPAPIEKTISKAKGQPREPQVYTKPPSREEMTKNQVSLKCLVKGFYPSDIAVEWESNGQPENNYKTTPPVLDSDGSFFLYSKLTVDKSRWQQGNVFSCSVMHEALHNHYTQKSLSLSPG

SEQ ID NO: 15 - protein, 329 aa, Homo sapiens
ASTKGPSVFPLAPSSKSTSGGTAALGCLVKDYFPEPVTVSWNSGALTSGVHTFPAVLQSSGLYSLSSVVTVPSSSLGTQTYICNVNHKPSNTKVDKRVEPKSCDKTHTCPPCPAPELGRGPSVFLFPPKPKDTLPISRTPEVTCVVVDVSHEDPEVKFNWYVDGVEVHNAKTKPREEQYNSTYRVVSVLTVLHQDWLNGKEYKCKVSNKALPAPIEKTISKAKGQPREPQVYTKPPSREEMTKNQVSLKCLVKGFYPSDIAVEWESNGQPENNYKTTPPVLDSDGSFFLYSKLTVDKSRWQQGNVFSCSVMHEALHNHYTQKSLSLSPG

SEQ ID NO: 16 - protein, 329 aa, Homo sapiens
ASTKGPSVFPLAPSSKSTSGGTAALGCLVKDYFPEPVTVSWNSGALTSGVHTFPAVLQSSGLYSLSSVVTVPSSSLGTQTYICNVNHKPSNTKVDKRVEPKSCDKTHTCPPCPAPELGRGPSVFLFPPKPKDTLRISRTPEVTCVVVDVSHEDPEVKFNWYVDGVEVHNAKTKPREEQYNSTYRVVSVLTVLHQDWLNGKEYKCKVSNKALPAPIEKTISKAKGQPREPQVYTKPPSREEMTKNQVSLKCLVKGFYPSDIAVEWESNGQPENNYKTTPPVLDSDGSFFLYSKLTVDKSRWQQGNVFSCSVMHEALHNHYTQKSLSLSPG

SEQ ID NO: 17 - protein, 329 aa, Homo sapiens
ASTKGPSVFPLAPSSKSTSGGTAALGCLVKDYFPEPVTVSWNSGALTSGVHTFPAVLQSSGLYSLSSVVTVPSSSLGTQTYICNVNHKPSNTKVDKRVEPKSCDKTHTCPPCPAPELGRGPSVFLFPPKPKDTLDISRTPEVTCVVVDVSHEDPEVKFNWYVDGVEVHNAKTKPREEQYNSTYRVVSVLTVLHQDWLNGKEYKCKVSNKALPAPIEKTISKAKGQPREPQVYTKPPSREEMTKNQVSLKCLVKGFYPSDIAVEWESNGQPENNYKTTPPVLDSDGSFFLYSKLTVDKSRWQQGNVFSCSVMHEALHNHYTQKSLSLSPG

SEQ ID NO: 18 - protein, 329 aa, Homo sapiens
ASTKGPSVFPLAPSSKSTSGGTAALGCLVKDYFPEPVTVSWNSGALTSGVHTFPAVLQSSGLYSLSSVVTVPSSSLGTQTYICNVNHKPSNTKVDKRVEPKSCDKTHTCPPCPAPELGRGPSVFLFPPKPKDTLMISRTPEVTCVVVDVSHEDPEVKFNWYVDGVEVHNAKTKPREEQYNSTYRVVSVLTVLHQDWLNGKEYKCKVSNKALPAPIEKTISKAKGQPREPQVYTKPPSREEMTKNQVSLKCLVKGFYPSDIAVEWESNGQPENNYKTTPPVLDSDGSFFLYSKLTVDKSRWQQGNVFSCSVMHEALHLHYTQKSLSLSPG

SEQ ID NO: 19 - protein, 329 aa, Homo sapiens
ASTKGPSVFPLAPSSKSTSGGTAALGCLVKDYFPEPVTVSWNSGALTSGVHTFPAVLQSSGLYSLSSVVTVPSSSLGTQTYICNVNHKPSNTKVDKRVEPKSCDKTHTCPPCPAPELGRGPSVFLFPPKPKDTLMISRTPEVTCVVVDVSHEDPEVKFNWYVDGVEVHNAKTKPREEQYNSTYRVVSVLTVLHQDWLNGKEYKCKVSNKALPAPIEKTISKAKGQPREPQVYTKPPSREEMTKNQVSLKCLVKGFYPSDIAVEWESNGQPENNYKTTPPVLDSDGSFFLYSKLTVDKSRWQQGNVFSCSVMHEALHNHYTEKSLSLSPG